European Patent Application EP 4 520 830 A1, published March 12, 2025. Title: Microorganism producing L-ornithine and L-ornithine production method using the same. Applicant: CJ CheilJedang Corporation. The sequence listing filed with the application follows.

SEQUENCE LISTING (34 sequences)

SEQ ID NO: 1 - protein, 205 aa, unidentified
  REGION 1..205: note = Shewanella corallii A687 LysE/ArgO family amino acid transporter AA
MQTAFIQGIGIGGSLIMAVGAQNAFVLKQGIKRSYPLPIAILCSIIDALMITAGVMGLGHLITSMPMIKHLASFGGAIFLIWYGANALRDSFRSKGLDLHQEQGADTLRKAVLTTLGISLLNPHLYLDTVVLLGSISTQFDDTVRPWFGAGAILASFLWFFSLSFGARLLGPLFEKPVAWRILDRFICLTMWSIAVALMWPYIKG

SEQ ID NO: 2 - DNA, 618 bp, unidentified
  misc_feature 1..618: note = Shewanella corallii A687 LysE/ArgO family amino acid transporter NT
  source 1..618: mol_type = genomic DNA
atgcagacagcatttattcaaggtataggtataggtggcagcctgatcatggctgttggtgcgcagaacgcgttcgtgctcaaacaggggattaaacgcagctatccgctgcccattgccattttgtgttcaatcatagacgcattgatgattactgccggtgtgatgggcctcgggcatttgatcaccagtatgcccatgattaagcatctggccagctttggtggtgccatattccttatctggtatggggctaatgcacttagagactccttcaggagcaaaggcctggatctgcaccaggagcagggggctgataccttgagaaaagcggtattgactacgcttgggatcagtttgctgaatccgcatctgtatctggatactgtggtgctgctgggcagtatcagtactcagtttgatgacacagtgcgtccctggtttggtgccggggctatattggcgtccttcctgtggttctttagcctgagctttggtgcacgcttgttgggacctttatttgaaaagccggtcgcgtggcggatattggacaggtttatctgtctgaccatgtggagtatcgcagtggccctgatgtggccatatattaaaggttga

SEQ ID NO: 3 - protein, 206 aa, unidentified
  REGION 1..206: note = Shewanella oneidensis MR-1 LysE/ArgO family amino acid transporter AA
MQTAFIQGMGIGGSLIIAVGAQNAFVLKQGIKRAYPLPIALLCSIIDALMITAGVAGLGHIIETFPTIKHVASFGGAAFLIWYGANALKASFVTKGMEMDHAQNADTLRKAILTTLGISLLNPHLYLDTVVLLGSISTQFEDAHRPWFGAGAVLASFIWFFSLSFGARLLAPIFSRPAAWRYLDRFIWLTMWSIAAAIIWPYLAAI

SEQ ID NO: 4 - DNA, 621 bp, unidentified
  misc_feature 1..621: note = Shewanella oneidensis MR-1 LysE/ArgO family amino acid transporter NT
  source 1..621: mol_type = genomic DNA
atgcaaacggcgtttattcaaggtatgggcattggtggtagtttgattattgccgtaggggcgcaaaatgctttcgtgctaaagcaagggattaagcgtgcttaccctttgccgattgcgctgctttgttcgattatcgatgccttgatgattaccgcgggtgtggcagggcttgggcatattattgagacctttccgaccattaagcacgtggcgagttttggtggtgcggcttttttgatttggtacggtgccaatgcgcttaaggcctcttttgttaccaaggggatggagatggatcacgcgcaaaatgctgatactctgcgtaaagccatcttgaccaccctaggcataagtctactcaatccacacctttatttagatactgtggtgttgcttggtagtatcagtactcagtttgaagatgctcaccgtccttggtttggcgccggtgcagtattggcttcttttatttggttctttagcctaagttttggtgcacgtttgttggcgcctatttttagtcgtccagcggcatggcgttatttagaccgctttatttggctgacgatgtggagcattgctgcggccattatctggccataccttgccgcaatttaa

SEQ ID NO: 5 - protein, 319 aa, unidentified
  REGION 1..319: note = ArgF WT AA
MTSQPQVRHFLADDDLTPAEQAEVLTLAAKLKAAPFSERPLEGPKSVAVLFDKTSTRTRFSFDAGIAHLGGHAIVVDSGSSQMGKGETLQDTAAVLSRYVEAIVWRTYAHSNFHAMAETSTVPLVNSLSDDLHPCQILADLQTIVENLSPEEGPAGLKGKKAVYLGDGDNNMANSYMIGFATAGMDISIIAPEGFQPRAEFVERAEKRGQETGAKVVVTDSLDEVAGADVVITDTWVSMGMENDGIDRTTPFVPYQVNDEVMAKANDGAIFLHCLPAYRGKEVAASVIDGPASKVFDEAENRLHAQKALLVWLLAHQPR

SEQ ID NO: 6 - DNA, 960 bp, unidentified
  misc_feature 1..960: note = argF WT NT
  source 1..960: mol_type = genomic DNA
atgacttcacaaccacaggttcgccatttcctggctgatgatgatctcacccctgcagagcaggcagaggttttgaccctagccgcaaagctcaaggcagcgccgttttcggagcgtccactcgagggaccaaagtccgttgcagttctttttgataagacttcaactcgtactcgcttctccttcgacgcgggcatcgctcatttgggtggacatgccatcgtcgtggattccggcagctcacagatgggtaagggcgagaccctgcaggacaccgcagctgtattgtcccgctacgtggaagcaattgtgtggcgcacctacgcacacagcaatttccacgccatggcggagacgtccactgtgccactggtgaactccttgtccgatgatctgcacccatgccagattctggctgatctgcagaccatcgtggaaaacctcagccctgaagaaggcccagcaggccttaagggtaagaaggctgtgtacctgggcgatggcgacaacaacatggccaactcctacatgattggctttgccaccgcgggcatggatatctccatcatcgctcctgaagggttccagcctcgtgcggaattcgtggagcgcgcggaaaagcgtggccaggaaaccggcgcgaaggttgttgtcaccgacagcctcgacgaggttgccggcgccgatgttgtcatcaccgatacctgggtatccatgggtatggaaaacgacggcatcgatcgcaccacacctttcgttccctaccaggtcaacgatgaggtcatggcgaaagctaacgacggcgccatcttcctgcactgccttcctgcctaccgcggcaaagaagtggcagcctccgtgattgatggaccagcgtccaaagttttcgatgaagcagaaaaccgcctccacgctcagaaagcactgctggtgtggctgctggcccaccagccgaggtaa

SEQ ID NO: 7 - protein, 171 aa, unidentified
  REGION 1..171: note = ArgR WT AA
MSLGSTPSTPENLNPVTRTARQALILQILDKQKVTSQVQLSELLLDEGIDITQATLSRDLDELGARKVRPDGGRAYYAVGPVDSIAREDLRGPSEKLRRMLDELLVSTDHSGNIAMLRTPPGAAQYLASFIDRVGLKEVVGTIAGDDTVFVLARDPLTGKELGELLSGRTT

SEQ ID NO: 8 - DNA, 516 bp, unidentified
  misc_feature 1..516: note = argR WT NT
  source 1..516: mol_type = genomic DNA
atgtcccttggctcaaccccgtcaacaccggaaaacttaaatcccgtgactcgcactgcacgccaagctctcattttgcagattttggacaaacaaaaagtcaccagccaggtacaactgtctgaattgctgctggatgaaggcatcgatatcacccaggccaccttgtcccgagatctcgatgaactcggtgcacgcaaggttcgccccgatgggggacgcgcctactacgcggtcggcccagtagatagcatcgcccgcgaagatctccggggtccgtcggagaagctgcgccgcatgcttgatgaactgctggtttctacagatcattccggcaacatcgcgatgctgcgcaccccgccgggagctgcccagtacctggcaagtttcatcgatagggtggggctgaaagaagtcgttggcaccatcgctggcgatgacaccgttttcgttctcgcccgtgatccgctcacaggtaaagaactaggtgaattactcagcgggcgcaccacttaa

SEQ ID NO: 9 - protein, 236 aa, unidentified
  REGION 1..236: note = LysE WT AA
MVIMEIFITGLLLGASLLLSIGPQNVLVIKQGIKREGLIAVLLVCLISDVFLFIAGTLGVDLLSNAAPIVLDIMRWGGIAYLLWFAVMAAKDAMTNKVEAPQIIEETEPTVPDDTPLGGSAVATDTRNRVRVEVSVDKQRVWVKPMLMAIVLTWLNPNAYLDAFVFIGGVGAQYGDTGRWIFAAGAFAASLIWFPLVGFGAAALSRPLSSPKVWRWINVVVAVVMTALAIKLMLMG

SEQ ID NO: 10 - DNA, 711 bp, unidentified
  misc_feature 1..711: note = lysE WT NT
  source 1..711: mol_type = genomic DNA
ctaacccatcaacatcagtttgatggccaatgcggtcatcacaactgccacgacgacgttgatccagcgccacaccttggggctggacagcgggcgtgacaatgctgctgcgccgaaacccaccagcgggaaccagatcaggcttgccgcgaacgcgccagcggcgaaaatccaccgtccggtgtcgccgtattgcgcgccgacgccgccgataaacacaaacgcgtccaaatacgcattcgggttcaaccaggtcagcacgattgccatcaacatgggcttcacccaaacccgctgcttatcgacgctcacctccacccgcacccggttgcgcgtgtcagtggccaccgccgaaccgcccaaaggcgtgtcatcgggcacggttggttctgtttcttcaatgatctgtggcgcttccaccttgtttgtcatggcgtctttcgctgccatgacggcaaaccataacaggtaagcgatgccaccccagcgcataatatcgagcacgatcggcgcggcattggacaaaagatcaacgcccaaggtgccggcgatgaacaaaaagacgtcagaaattaaacacacgagaagaaccgcaatgagtccttcgcgcttaattccttgtttaatcaccagtacattctgcggtccgatggacagcaaaagactggcccccaaaagcagacctgtaatgaagatttccatgatcaccat

SEQ ID NO: 11 - DNA, 35 bp, synthetic construct
  misc_feature 1..35: note = primer 1
  source 1..35: mol_type = other DNA
cggtacccggggatccttttagattcccagtgcag

SEQ ID NO: 12 - DNA, 20 bp, synthetic construct
  misc_feature 1..20: note = primer 2
  source 1..20: mol_type = other DNA
cgcgtgggctttgggctgag

SEQ ID NO: 13 - DNA, 20 bp, synthetic construct
  misc_feature 1..20: note = primer 3
  source 1..20: mol_type = other DNA
tgcattggtggagctagctg

SEQ ID NO: 14 - DNA, 35 bp, synthetic construct
  misc_feature 1..35: note = primer 4
  source 1..35: mol_type = other DNA
atgcctgcaggtcgacgctatgcagtggagatgtc

SEQ ID NO: 15 - DNA, 37 bp, synthetic construct
  misc_feature 1..37: note = primer 5_ Sco
  source 1..37: mol_type = other DNA
ctttagaggagacacaacatgcagacagcatttattc

SEQ ID NO: 16 - DNA, 35 bp, synthetic construct
  misc_feature 1..35: note = primer 6_ Sco
  source 1..35: mol_type = other DNA
tagctccaccaatgcatcaacctttaatatatggc

SEQ ID NO: 17 - DNA, 37 bp, synthetic construct
  misc_feature 1..37: note = primer 5_Son
  source 1..37: mol_type = other DNA
ctttagaggagacacaacatgcaaacggcgtttattc

SEQ ID NO: 18 - DNA, 35 bp, synthetic construct
  misc_feature 1..35: note = primer 6_Son
  source 1..35: mol_type = other DNA
tagctccaccaatgcattaaattgcggcaaggtat

SEQ ID NO: 19 - DNA, 35 bp, synthetic construct
  misc_feature 1..35: note = primer 7
  source 1..35: mol_type = other DNA
gcccaaagcccacgcgaacgaccgagcctattggg

SEQ ID NO: 20 - DNA, 22 bp, synthetic construct
  misc_feature 1..22: note = primer 8
  source 1..22: mol_type = other DNA
gttgtgtctcctctaaagattg

SEQ ID NO: 21 - DNA, 20 bp, synthetic construct
  misc_feature 1..20: note = primer 9
  source 1..20: mol_type = other DNA
tattacgccagctggcgaaa

SEQ ID NO: 22 - DNA, 20 bp, synthetic construct
  misc_feature 1..20: note = primer 10
  source 1..20: mol_type = other DNA
gctttacactttatgcttcc

SEQ ID NO: 23 - DNA, 35 bp, synthetic construct
  misc_feature 1..35: note = primer 11
  source 1..35: mol_type = other DNA
cggtacccggggatcctgaccccaggcaagcacgg

SEQ ID NO: 24 - DNA, 27 bp, synthetic construct
  misc_feature 1..27: note = primer 12
  source 1..27: mol_type = other DNA
gaagcgagtacgagtttaagtcttatc

SEQ ID NO: 25 - DNA, 20 bp, synthetic construct
  misc_feature 1..20: note = primer 13
  source 1..20: mol_type = other DNA
aaactcgtactcgcttctcc

SEQ ID NO: 26 - DNA, 35 bp, synthetic construct
  misc_feature 1..35: note = primer 14
  source 1..35: mol_type = other DNA
atgcctgcaggtcgaccggcgccggcaacctcgtc

SEQ ID NO: 27 - DNA, 36 bp, synthetic construct
  misc_feature 1..36: note = primer 15
  source 1..36: mol_type = other DNA
cggtacccggggatccctcgtgcggaattcgtggag

SEQ ID NO: 28 - DNA, 20 bp, synthetic construct
  misc_feature 1..20: note = primer 16
  source 1..20: mol_type = other DNA
atccagcagcaattcagaca

SEQ ID NO: 29 - DNA, 37 bp, synthetic construct
  misc_feature 1..37: note = primer 17
  source 1..37: mol_type = other DNA
ctgaattgctgctggattaaggcatcgatatcaccca

SEQ ID NO: 30 - DNA, 36 bp, synthetic construct
  misc_feature 1..36: note = primer 18
  source 1..36: mol_type = other DNA
atgcctgcaggtcgacccttcattttaagttccttg

SEQ ID NO: 31 - DNA, 36 bp, synthetic construct
  misc_feature 1..36: note = primer 19
  source 1..36: mol_type = other DNA
cggtacccggggatccattgcctcaccaaaaccttc

SEQ ID NO: 32 - DNA, 23 bp, synthetic construct
  misc_feature 1..23: note = primer 20
  source 1..23: mol_type = other DNA
cgtgacctatggaagtacttaag

SEQ ID NO: 33 - DNA, 38 bp, synthetic construct
  misc_feature 1..38: note = primer 21
  source 1..38: mol_type = other DNA
gtacttccataggtcacgttagttttcgcgggttttag

SEQ ID NO: 34 - DNA, 36 bp, synthetic construct
  misc_feature 1..36: note = primer 22
  source 1..36: mol_type = other DNA
atgcctgcaggtcgacgttttggtggttcccgaaag